European Patent Application EP 4 246 143 A1, published September 20, 2023. Title: In-vitro method for diagnosis of pemphigus vulgaris in a patient and/or of determining disease activity in a pemphigus vulgaris patient. Applicant: Philipps-Universität Marburg. The sequence listing filed with the application follows.

SEQUENCE LISTING (9 sequences)

SEQ ID NO: 1 - protein, 15 aa, Homo sapiens
LNSKIAFKIVSQEPA

SEQ ID NO: 2 - protein, 15 aa, Homo sapiens
TPMFLLSRNTGEVRT

SEQ ID NO: 3 - protein, 15 aa, Homo sapiens
CECNIKVKDVNDNFP

SEQ ID NO: 4 - protein, 17 aa, Homo sapiens
INVREGIAFRPASKTFT

SEQ ID NO: 5 - protein, 15 aa, Homo sapiens
LNSKIAFKIVSQEPA

SEQ ID NO: 6 - protein, 15 aa, Homo sapiens
TPMFLLSRNTGEVRT

SEQ ID NO: 7 - protein, 15 aa, Homo sapiens
NIKVKDVNDNFPMFR

SEQ ID NO: 8 - protein, 15 aa, Homo sapiens
REGIAFRPASKTFTV

SEQ ID NO: 9 - protein, 566 aa, Homo sapiens
MMGLFPRTTGALAIFVVVILVHGELRIETKGQYDEEEMTMQQAKRRQKREWVKFAKPCREGEDNSKRNPIAKITSDYQATQKITYRISGVGIDQPPFGIFVVDKNTGDINITAIVDREETPSFLITCRALNAQGLDVEKPLILTVKILDINDNPPVFSQQIFMGEIEENSASNSLVMILNATDADEPNHLNSKIAFKIVSQEPAGTPMFLLSRNTGEVRTLTNSLDREQASSYRLVVSGAWLAVYFFTSGNEGNWFEIQTDPRTNEGILKVVKALDYEQLQSVKLSIAVKNKAEFHQSVISRYRVQSTPVTIQVINVREGIAFRPASKTFTVQKGISSKKLVDYILGTYQAIDEDTNKAAVYVRVPDFNDNCPTAVLEDKAVCSSSPSVVVSARTLNNRYTGPYTFALEDQPVKLPAVWSSNVKYVMGRNDGGYMLMIDSKTAEIKFVKNMNRDSTFIVNKTITAEVLAIDEYTGKTSTGVYVRVPDFNDNCPTAVLEKDAVCSSSPSVVVSARTLNNRYTGPYTFALEDQPVKLPAVWSITTLNATSALLRAQEQIPPGVYHISL